European Patent Specification EP 3 436 005 B1, published January 28, 2026. Title: CALCIUM SENSING RECEPTORS, LIGANDS, COMPOSITIONS, AND METHODS OF USE. Applicant: Georgia Sate University Research Foundation, Inc. The sequence listing filed with the application follows.

SEQUENCE LISTING (18 sequences)

SEQ ID NO: 1 - protein, 593 aa, Homo sapiens
YGPDQRAQKKGDIILGGLFPIHFGVAAKDQDLKSRPESVECIRYNFRGFRWLQAMIFAIEEINSSPALLPNLTLGYRIFDTCNTVSKALEATLSFVAQNKIDSLNLDEFCNCSEHIPSTIAVVGATGSGVSTAVANLLGLFYIPQVSYASSSRLLSNKNQFKSFLRTIPNDEHQATAMADIIEYFRWNWVGTIAADDDYGRPGIEKFREEAEERDICIDFSELISQYSDEEEIQHVVEVIQNSTAKVIVVFSSGPDLEPLIKEIVRRNITGKIWLASEAWASSSLIAMPQYFHVVGGTIGFALKAGQIPGFREFLKKVHPRKSVHNGFAKEFWEETFNCHLQEGAKGPLPVDTFLRGHEESGDRFSNSSTAFRPLCTGDENISSVETPYIDYTHLRISYNVYLAVYSIAHALQDIYTCLPGRGLFTNGSCADIKKVEAWQVLKHLRHLNFTNNMGEQVTFDECGDLVGNYSIINWHLSPEDGSIVFKEVGYYNVYAKKGERLFINEEKILWSGFSREVPFSNCSRDCLAGTRKGIIEGEPTCCFECVECPDGEYSDETDASACNKCPDDFWSNENHTSCIAKEIEFLSWTEPF

SEQ ID NO: 2 - protein, 600 aa, Artificial Sequence
  human CaSR with FLAG Tag
YGPDQRAQKKGDIILGGLFPIHFGVAAKDQDLKSRPESVECIRYNFRGFRWLQAMIFAIEEINSSPALLPNLTLGYRIFDTCNTVSKALEATLSFVAQNKIDSLNLDEFCNCSEHIPSTIAVVGATGSGVSTAVANLLGLFYIPQVSYASSSRLLSNKNQFKSFLRTIPNDEHQATAMADIIEYFRWNWVGTIAADDDYGRPGIEKFREEAEERDICIDFSELISQYSDEEEIQHVVEVIQNSTAKVIVVFSSGPDLEPLIKEIVRRNITGKIWLASEAWASSSLIAMPQYFHVVGGTIGFALKAGQIPGFREFLKKVHPRKSVHNGFAKEFWEETFNCHLQEGAKGPLPVDYKDDDDKTFLRGHEESGDRFSNSSTAFRPLCTGDENISSVETPYIDYTHLRISYNVYLAVYSIAHALQDIYTCLPGRGLFTNGSCADIKKVEAWQVLKHLRHLNFTNNMGEQVTFDECGDLVGNYSIINWHLSPEDGSIVFKEVGYYNVYAKKGERLFINEEKILWSGFSREVPFSNCSRDCLAGTRKGIIEGEPTCCFECVECPDGEYSDETDASACNKCPDDFWSNENHTSCIAKEIEFLSWTEPF

SEQ ID NO: 3 - protein, 169 aa, Artificial Sequence
  ECD subdomain 1 of CaSR (amino acids 132-300 of SEQ ID NO: 1)
SEHIPSTIAVVGATGSGVSTAVANLLGLFYIPQVSYASSSRLLSNKNQFKSFLRTIPNDEHQATAMADIIEYFRWNWVGTIAADDDYGRPGIEKFREEAEERDICIDFSELISQYSDEEEIQHVVEVIQNSTAKVIVVFSSGPDLEPLIKEIVRRNITGKIWLASEAWA

SEQ ID NO: 4 - protein, 140 aa, Artificial Sequence
  ECD subdomain 2 of CaSR (amino acids 185-324 of SEQ ID NO: 1)
RTIPNDEHQATAMADIIEYFRWNWVGTIAADDDYGRPGIEKFREEAEERDICIDFSELISQYSDEEEIQHVVEVIQNSTAKVIVVFSSGPDLEPLIKEIVRRNITGKIWLASEAWASSSLIAMPQYFHVVGGTIGFALKA

SEQ ID NO: 5 - protein, 106 aa, Artificial Sequence
  ECD subdomain 3 of human CaSR (amino acids 340-445 of SEQ ID NO: 1)
RKSVHNGFAKEFWEETFNCHLQEGAKGPLPVDTFLRGHEESGDRFSNSSTAFRPLCTGDENISSVETPYIDYTHLRISYNVYLAVYSIAHALQDIYTCLPGRGLFT

SEQ ID NO: 6 - protein, 84 aa, Artificial Sequence
  human CaSR systeine rich domain
LWSGFSREVPFSNCSRDCLAGTRKGIIEGEPTCCFECVECPDGEYSDETDASACNKCPDDFWSNENHTSCIAKEIEFLSWTEPF

SEQ ID NO: 7 - protein, 688 aa, Artificial Sequence
  Shark CaSR ECD
MVFPSPFGPCCQLVLRWKTSKENRCSSLKVSTTESAPTITETSKKAQTFVSKLTLVEAEQSDLLKALGEEDCTMGGHHYGLLILGFTLLQSYCVSEYGPNQRAQKKGDIILGGLFPIHFGVTAKDQDLKSRPEMTKCFRYNFRGFRWLQAMIFAIEEINNSMAFLPNITLGYRIFDTCNTVSKALEATLSFVAQNKIDSLNLDEFCNCSDHIPSTIAVVGATGSGISTAVANLLGLFYIPQVSYASSSRLLSNKNQYKSFLRTIPNDEQQATAMADIIQHFQWNWVGTLAADDDYGRPGIEKFREEAEERDICIDFSELISQYYTQEELQHVAEVIQNSTAKVIVVFSSGPDLEPIIQEIVRRNITGRIWLASEAWASSSLIAKPEYFHVVGGTIGFALRAGHIPGFYEFLQRVHPSRSSDNGFVKEFWEETFKCYLTEKSLTQLKQSKTPGHDGSTVVGNITSSKLLPPCTGDENIMSVETPYLDYTHMRISYNVYMAVYSIAHALQDIYTCTPGKGIFENGSCADIKKVEAWQVLKHLKHLKFTNSMGEQVDFDDQGDLKGNYTIINWQLSSEDQSVVFQEVGNYNAYAKPGERLYINESKVLWSGFSKVVPFSNCTHDCIPGTRKGIIEGEPTCCFECVSCAEGEYSDENDASACTKCPNDFWSNENHTYCIEKEIEYLSWTEPF

SEQ ID NO: 8 - protein, 601 aa, Artificial Sequence
  Zebrafish CaSR ECD
MRFHLKFYLHYLVLLGSSCVISTYGPNQRAQKTGDILLGGLFPMHFGVASKDQDLAARPESTECVRYNFRGFRWLQSMIFAIEEINNSSTLLPNITLGYRIFDTCNTVSKALEASLSFVAQNKIDSLNLDEFCNCTGNIPSTIAVVGASGSAVSTAVADLLGLFYIPQISYASSSRLLSNKNQYKSFMRTIPTDEYQAIAMAAIIEHFQWNWVIAIASDDEYGRPGIEKFENEMFHRDICIDLNVLISQYVDEAEIRRLADRIQNSSAKVIVVFASGPDIEPLVKEMVRRNITDRVWLASEAWASSSLVAKPEYLDVMGGTIGFALRAGHIPGFKDFLQQVHPKKSSHNEFVREFWEETFNCYLEDSPRNADSENGSTSFRPLCTGEEDIASVETPYLDYTHLRISYNVYVAVYAIAQALQDILTCTPGKGLFSNGSCADIRKVEAWQVLKQLRHLNFIDSMGERVRFDNGSELSANYTIINWHRSPEDGSVVFKEVGYYSIHNKNVAKLSIDKSKILWNGRLTEVPFSNCSVECEPGTRKGIIDGEPTCCFECTECSDGEYSDHKDASFCVKCPNNSWSNGNHTSCFLKQIEFLSWTEPF

SEQ ID NO: 9 - protein, 597 aa, Artificial Sequence
  Salmon CaSR ECD
MRFYLYYLVLLGFSSVISTYGPHQRAQKTGDILLGGLFPMHFGVTSKDQDLAARPESTECVRYNFRGFRWLQAMIFAIEEINNSSTLLPNITLGYRIFDTCNTVSKALEATLSFVAQNKIDSLNLDEFCNCTDHIPSTIAVVGASGSAVSTAVANLLGLFYIPQISYASSSRLLSNKNQFKSFMRTIPTDEHQATAMADIIDYFQWNWVIAVASDDEYGRPGIEKFEKEMEERDICIHLSELISQYFEEWQIQGLVDRIENSSAKVIVVFASGPDIEPLIKEMVRRNITDRIWLASEAWATTSLIAKPEYLDVVVGTIGFALRAGEIPGFKDFLQEVTPKKSSHNEFVREFWEETFNCYLEDSQRLRDSENGSTSFRPLCTGEEDIMGAETPYLDYTHLRISYNVYVAVHSIAQALQDILTCIPGRGLFSNNSCADIKKIEAWQVLKQLRHLNFSNSMGEKVHFDENADPSGNYTIINWHRSPEDGSVVFEEVGFYNMRAKRGVQLFIDNTKILWNGYNTEVPFSNCSEDCEPGTRKGIIESMPTCCFECTECSEGEYSDHKDASVCTKCPNDSWSNENHTSCFLKEIEFLSWTEPF

SEQ ID NO: 10 - protein, 611 aa, Artificial Sequence
  Chicken CaSR ECD
MTLYSCCLILLLFTWNTAAYGPNQRAQKKGDIILGGLFPIHFGVAAKDQDLKSRPESVECIRYNFRGFRWLQAMIFAIEEINNSPNLLPNMTLGYRIFDTCNTVSKALEATLSFVAQNKIDSLNLDEFCNCSEHIPSTIAVVGATGSGVSTAVANLLGLFYIPQVSYASSSRLLSNKNQFKSFLRTIPNDEHQATAMADIIEYFRWNWVGTIAADDDYGRPGIEKFREEAEERDICIDFSELISQYSDEEEIQQVVEVIQNSTARVIVVFSSGPDLEPLIKEIVRRNITGKIWLASEAWASSSLIAMPEFFRVIGSTIGFALKAGQIPGFREFLQKVHPKKSANNGFAKEFWEETFNCYLPSESKNSPASASFHKAHEEGLGAGNGTAAFRPPCTGDENITSVETPYMDFTHLRISYNVYLAVYSIAHALQDIYTCTPGKGLFTNGSCADIKKVEAWQVLKHLRHLNFTSNMGEQVDFDEFGDLVGNYSIINWHLSPEDGSVVFEEVGHYNVYAKKGERLFINENKILWSGFSKEVPFSNCSRDCLPGTRKGIIEGEPTCCFECVDCPDGEYSDETDASACDKCPEDYWSNENHTSCIPKQIEFLSWTEPF

SEQ ID NO: 11 - protein, 612 aa, Artificial Sequence
  Mouse CaSR ECD
MAWFGYCLALLALTWHSSAYGPDQRAQKKGDIILGGLFPIHFGVSAKDQDLKSRPESVECIRYNFRGFRWLQAMIFAIEEINSSPALLPNMTLGYRIFDTCNTVSKALEATLSFVAQNKIDSLNLDEFCNCSEHIPSTIAVVGATGSGVSTAVANLLGLFYIPQVSYASSSRLLSNKNQFKSFLRTIPNDEHQATAMADIIEYFRWNWVGTIAADDDYGRPGIEKFREEAEERDICIDFSELISQYSDEEEIQQVVEVIQNSTAKVIVVFSSGPDLEPLIKEIVRRNITGRIWLASEAWASSSLIAMPEYFHVVGGTIGFGLKAGQIPGFREFLQKVHPRKSVHNGFAKEFWEETFNCHLQDGAKGPLPVDTFVRSHEEGGNRLLNSSTAFRPLCTGDENINSVETPYMDYEHLRISYNVYLAVYSIAHALQDIYTCLPGRGLFTNGSCADIKKVEAWQVLKHLRHLNFTNNMGEQVTFDECGDLVGNYSIINWHLSPEDGSIVFKEVGYYNVYAKKGERLFINEGKILWSGFSREVPFSNCSRDCQAGTRKGIIEGEPTCCFECAECPDGEYSGETDASACDKCPDDFWSNENHTSCIAKEIEFLAWTEPF

SEQ ID NO: 12 - protein, 612 aa, Artificial Sequence
  Rat CaSR ECD
MASYSCCLALLALAWHSSAYGPDQRAQKKGDIILGGLFPIHFGVAAKDQDLKSRPESVECIRYNFRGFRWLQAMIFAIEEINSSPSLLPNMTLGYRIFDTCNTVSKALEATLSFVAQNKIDSLNLDEFCNCSEHIPSTIAVVGATGSGVSTAVANLLGLFYIPQVSYASSSRLLSNKNQYKSFLRTIPNDEHQATAMADIIEYFRWNWVGTIAADDDYGRPGIEKFREEAEERDICIDFSELISQYSDEEEIQQVVEVIQNSTAKVIVVFSSGPDLEPLIKEIVRRNITGRIWLASEAWASSSLIAMPEYFHVVGGTIGFGLKAGQIPGFREFLQKVHPRKSVHNGFAKEFWEETFNCHLQEGAKGPLPVDTFVRSHEEGGNRLLNSSTAFRPLCTGDENINSVETPYMDYEHLRISYNVYLAVYSIAHALQDIYTCLPGRGLFTNGSCADIKKVEAWQVLKHLRHLNFTNNMGEQVTFDECGDLVGNYSIINWHLSPEDGSIVFKEVGYYNVYAKKGERLFINEEKILWSGFSREVPFSNCSRDCQAGTRKGIIEGEPTCCFECVECPDGEYSGETDASACDKCPDDFWSNENHTSCIAKEIEFLAWTEPF

SEQ ID NO: 13 - protein, 612 aa, Artificial Sequence
  human CasR ECD
MAFYSCCWVLLALTWHTSAYGPDQRAQKKGDIILGGLFPIHFGVAAKDQDLKSRPESVECIRYNFRGFRWLQAMIFAIEEINSSPALLPNLTLGYRIFDTCNTVSKALEATLSFVAQNKIDSLNLDEFCNCSEHIPSTIAVVGATGSGVSTAVANLLGLFYIPQVSYASSSRLLSNKNQFKSFLRTIPNDEHQATAMADIIEYFRWNWVGTIAADDDYGRPGIEKFREEAEERDICIDFSELISQYSDEEEIQHVVEVIQNSTAKVIVVFSSGPDLEPLIKEIVRRNITGKIWLASEAWASSSLIAMPQYFHVVGGTIGFALKAGQIPGFREFLKKVHPRKSVHNGFAKEFWEETFNCHLQEGAKGPLPVDTFLRGHEESGDRFSNSSTAFRPLCTGDENISSVETPYIDYTHLRISYNVYLAVYSIAHALQDIYTCLPGRGLFTNGSCADIKKVEAWQVLKHLRHLNFTNNMGEQVTFDECGDLVGNYSIINWHLSPEDGSIVFKEVGYYNVYAKKGERLFINEEKILWSGFSREVPFSNCSRDCLAGTRKGIIEGEPTCCFECVECPDGEYSDETDASACNKCPDDFWSNENHTSCIAKEIEFLSWTEPF

SEQ ID NO: 14 - protein, 622 aa, Artificial Sequence
  gibbon CaSR ECD
MAFYSCCWVLLALTWHTSAYGPDQRAQKKGDIILGGLFPIHFGVAAKDQDLKSRPESVECIRYNFRGFRWLQAMIFAIEEINSSPALLPNLTLGYRIFDTCNTVSKALEATLSFVAQNKIDSLNLDEFCNCSEHIPSTIAVVGATGSGVSTAVANLLGLFYIPQVSYASSSRLLSNKNQFKSFLRTIPNDEHQATAMADIIEYFRWNWVGTIAADDDYGRPGIEKFREEAEERDICIDFSELISQYSDEEEIQHVVEVIQNSTAKVIVVFSSGPDLEPLIKEIVRRNITGKIWLASEAWASSSLIAMPQYFHVVGGTIGFALKAGQIPGFREFLKKVHPRKSVHNGFAKEFWEETFNCHLQEGAKGPLPVDTFLRGHEESGGRFSNSSTAFRPLCTGDENISSVETPYIDYTHLRISYNVYLAVYSIAHALQDIYTCLPGRGLFTNGSCADIKKVEAWQVLKHLRHLNFTNNMGEQVTFDECGDLVGNYSIINWHLSAEDGSIVFKEVGYYNVYAKKGERLFINEEKILWSGFSREPLTFVLSVPQVPFSNCSRDCLAGTRKGIIEGEPTCCFECVECPDGEYSDETDASACNKCPDDFWSNENHTSCIAKEIEFLSWTEPF

SEQ ID NO: 15 - protein, 612 aa, Artificial Sequence
  dog CaSR ECD
MAFHSCSLILLAITWCTSAYGPDQRAQKKGDIILGGLFPIHFGVAAKDQDLKSRPESVECIRYNFRGFRWLQAMIFAIEEINSSPALLPNMTLGYRIFDTCNTVSKALEATLSFVAQNKIDSLNLDEFCNCSEHIPSTIAVVGATGSGISTAVANLLGLFYIPQVSYASSSRLLSNKNQFKSFLRTIPNDEHQATAMADIIEYFRWNWVGTIAADDDYGRPGIEKFREEAEERDICIDFSELISQYSDEEEIQQVVEVIQNSTAKVIVVFSSGPDLEPLIKEIVRRNITGRIWLASEAWASSSLIAMPEYFHVVGGTIGFALKAGQIPGFREFLQKVHPRKSVHNGFAKEFWEETFNCHLQEGAKGPLSMDTFLRGHEEGGGRISNSSTAFRPLCTGDENISSVETPYMDYTHLRISYNVYLAVYSIAHALQDIYTCLPGRGLFTNGSCADIKKVEAWQVLKHLRHLNFTNNMGEQVTFDECGDLMGNYSIINWHLSPEDGSIVFKEVGYYNVYAKKGERLFINEEKILWSGFSREMPFSNCSRDCLAGTRKGIIEGEPTCCFECVECPDGEYSDETDASACDKCPDDFWSNENHTSCIAKEIEFLSWTEPF

SEQ ID NO: 16 - protein, 553 aa, Artificial Sequence
  Bovine CaSR ECD
MALYSCCWILLAFSTWCTSAYGPDQRAQKKGDIILGGLFPIHFGVAVKDQDLKSRPESVECIRYNFRGFRWLQAMIFAIEEINSSPALLPNMTLGYRIFDTCNTQVSYASSSRLLSNKNQFKSFLRTIPNDEHQATAMADIIEYFRWNWVGTIAADDDYGRPGIEKFREEAEERDICIDFSELISQYSDEEKIQQVVEVIQNSTAKVIVVFSSGPDLEPLIKEIVRRNITGRIWLASEAWASSSLIAMPEYFHVVGGTIGFGLKAGQIPGFREFLQKVHPRKSVHNGFAKEFWEETFNCHLQEGAKGPLPVDTFLRGHEEGGARLSNSPTAFRPLCTGEENISSVETPYMDYTHLRISYNVYLAVYSIAHALQDIYTCIPGRGLFTNGSCADIKKVEAWQVLKHLRHLNFTSNMGEQVTFDECGDLAGNYSIINWHLSPEDGSIVFKEVGYYNVYAKKGERLFINDEKILWSGFSREVPFSNCSRDCLAGTRKGIIEGEPTCCFECVECPDGEYSDETDASACDKCPDDFWSNENHTSCIAKEIEFLSWTEPF

SEQ ID NO: 17 - protein, 612 aa, Artificial Sequence
  Alpaca CaSR ECD
MASYSCCWILLAFAWCASAYGPDQRAQKKGDIILGGLFPIHFGVAAKDQDLKSRPESVECIRYNFRGFRWLQAMIFAIEEINSSPALLPNMTLGYRIFDTCNTVSKALEATLSFVAQNKIDSLNLDEFCNCSEHIPSTIAVVGATGSGISTAVANLLGLFYIPQVSYASSSRLLSNKNQFKSFLRTIPNDEHQATAMADIIEYFRWNWVGTIAADDDYGRPGIEKFREEAEERDICIDFSELISQYSDEEEIQQVVEVIQNSTAKVIVVFSSGPDLEPLIKEIVRRNITGRIWLASEAWASSSLIAMPEYFHVVGGTIGFALKAGQIPGFREFLQKVHPRKSVHNGFAKEFWEETFNCHLQEGAKGPLPVDNFLRGHEEGGGRTSNSSTAFRPLCTGDENISSVETPYMDYTHLRISYNVYLAVYSIAHALQDIYTCIPGRGLFTNGSCADIKKVEAWQVLKHLRHLNFTNNMGEQVTFDECGDLAGNYSIINWHLSPEDGSIVFKEVGYYNVYAKKGERLFINEEKILWSGFSREVPFSNCSRDCLAGTRKGIIEGEPTCCFECVECPDGEYSDETDASACDKCPDDFWSNENHTSCIAKEIEFLSWTEPF

SEQ ID NO: 18 - protein, 622 aa, Artificial Sequence
  pig CaSR ECD
MAFSSCCWILLALTWCTSAYGPDQRAQKKGDIILGGLFPIHFGVAAKDQNLESRPESVECIRYNFRGFRWLQAMIFAIEEINSSPALLPNMTLGYRIFDTCNTVSKALEATLSFVAQNKIDSLNLDEFCNCSEHIPSTIAVVGATGSGISTAVANLLGLFYIPQVSYASSSRLLSNKNQFKSFLRTIPNDEHQATAMADIIEYFRWNWVGTIAADDDYGRPGIEKFREEAEERDICIDFSELISQYSDEEEIQQVVEVIQNSTAKVIVVFSSGPDLEPLIKEIVRRNITGKIWLASEAWASSSLIAMPEYFHVVGGTIGFALKAGQIPGFREFLQKVHPSKSVHNGFAKEFWEETFNCHLQEGAKGPLTTDTFLRGHEEGGGRISNSSTAFRPLCTGDENISSVETPYMDYTHLRISYNVYLAVYSIAHALQDIYTCIPGRGLFTNGSCADIKKVEAWQVLKHLRHLNFTSNMGEQVTFDEYGDLAGNYSIINWHLSPEDGSIVFKEVGYYNVYAKKGERLFINEEKILWSGFSREPLTVVLPILQVPFSNCSRDCLAGTRKGIIEGEPTCCFECVECPDGEYSDETDASACDKCPDDFWSNENHTSCIAKEIEFLSWTEPF